European Patent Application EP 4 606 817 A1, published August 27, 2025. Title: MANUFACTURE AND APPLICATION OF FLAGELLIN IMMUNOPOTENTIATING DERIVATIVES WITH TLR5 ACTIVITY USING EUKARYOTIC CELL EXPRESSION SYSTEMS. Applicant: INDUSTRY FOUNDATION OF CHONNAM NATIONAL UNIVERSITY. Application KR PCT/KR2023/010821, filed July 26, 2023. The sequence listing filed with the application follows.

SEQUENCE LISTING (23 sequences)

SEQ ID NO: 1 - DNA, 29 bp, synthetic construct
  source 1..29: mol_type = other DNA
cccaagcttgccgtcaacgtgaacaccaa

SEQ ID NO: 2 - DNA, 36 bp, synthetic construct
  source 1..36: mol_type = other DNA
atagtttagcggccgcgcccagcagggagagggcgc

SEQ ID NO: 3 - DNA, 32 bp, synthetic construct
  source 1..32: mol_type = other DNA
ctgaaggcgccatggccgaaaccaccaacatc

SEQ ID NO: 4 - DNA, 32 bp, synthetic construct
  source 1..32: mol_type = other DNA
gatgttggtggtttcggccatggcgccttcag

SEQ ID NO: 5 - DNA, 32 bp, synthetic construct
  source 1..32: mol_type = other DNA
ctctgcagtctgccgccggcagcaacagcaag

SEQ ID NO: 6 - DNA, 32 bp, synthetic construct
  source 1..32: mol_type = other DNA
cttgctgttgctgccggcggcagactgcagag

SEQ ID NO: 7 - DNA, 30 bp, synthetic construct
  source 1..30: mol_type = other DNA
caacaagctgctggctggcacctacggcac

SEQ ID NO: 8 - DNA, 30 bp, synthetic construct
  source 1..30: mol_type = other DNA
gtgccgtaggtgccagccagcagcttgttg

SEQ ID NO: 9 - DNA, 30 bp, synthetic construct
  source 1..30: mol_type = other DNA
gggcgagggcaaggccgtgaccgtggatac

SEQ ID NO: 10 - DNA, 30 bp, synthetic construct
  source 1..30: mol_type = other DNA
gtatccacggtcacggccttgccctcgccc

SEQ ID NO: 11 - DNA, 31 bp, synthetic construct
  source 1..31: mol_type = other DNA
caacgagaacgtcgctgcctctaagtccagg

SEQ ID NO: 12 - DNA, 31 bp, synthetic construct
  source 1..31: mol_type = other DNA
cctggacttagaggcagcgacgttctcgttg

SEQ ID NO: 13 - protein, 377 aa, synthetic construct
MAVNVNTNVAAMTAQRYLNNANSAQQTSMERLSSGFKINSAKDDAAGLQISNRLNVQSRGLDVAVRNANDGISIAQTAEGAMNETTNILQRMRDLSLQSANGSNSKSERVAIQEEVTALNDELNRIAETTSFGGNKLLNGTYGTKAMQIGADNGEAVMLSLKDMRSDNVMMGGVSYQAEEGKDKNWNVAAGDNDLTIALTDSFGNEQEIEINAKAGDDIEELATYINGQTDLVKASVGEGGKLQIFAGNNKVQGEIAFSGSLAGELGLGEGKNVTVDTIDVTTVQGAQESVAIVDAALKYVDSHRAELGAFQNRFNHAISNLDNINENVNASKSRIKDTDFAKETTQLTKTQILSQASSSILAQAKQAPNSALSLLG

SEQ ID NO: 14 - protein, 377 aa, synthetic construct
MAVNVNTNVAAMTAQRYLNNANSAQQTSMERLSSGFKINSAKDDAAGLQISNRLNVQSRGLDVAVRNANDGISIAQTAEGAMAETTNILQRMRDLSLQSANGSNSKSERVAIQEEVTALNDELNRIAETTSFGGNKLLNGTYGTKAMQIGADNGEAVMLSLKDMRSDNVMMGGVSYQAEEGKDKNWNVAAGDNDLTIALTDSFGNEQEIEINAKAGDDIEELATYINGQTDLVKASVGEGGKLQIFAGNNKVQGEIAFSGSLAGELGLGEGKNVTVDTIDVTTVQGAQESVAIVDAALKYVDSHRAELGAFQNRFNHAISNLDNINENVNASKSRIKDTDFAKETTQLTKTQILSQASSSILAQAKQAPNSALSLLG

SEQ ID NO: 15 - protein, 377 aa, synthetic construct
MAVNVNTNVAAMTAQRYLNNANSAQQTSMERLSSGFKINSAKDDAAGLQISNRLNVQSRGLDVAVRNANDGISIAQTAEGAMNETTNILQRMRDLSLQSAAGSNSKSERVAIQEEVTALNDELNRIAETTSFGGNKLLNGTYGTKAMQIGADNGEAVMLSLKDMRSDNVMMGGVSYQAEEGKDKNWNVAAGDNDLTIALTDSFGNEQEIEINAKAGDDIEELATYINGQTDLVKASVGEGGKLQIFAGNNKVQGEIAFSGSLAGELGLGEGKNVTVDTIDVTTVQGAQESVAIVDAALKYVDSHRAELGAFQNRFNHAISNLDNINENVNASKSRIKDTDFAKETTQLTKTQILSQASSSILAQAKQAPNSALSLLG

SEQ ID NO: 16 - protein, 377 aa, synthetic construct
MAVNVNTNVAAMTAQRYLNNANSAQQTSMERLSSGFKINSAKDDAAGLQISNRLNVQSRGLDVAVRNANDGISIAQTAEGAMNETTNILQRMRDLSLQSANGSNSKSERVAIQEEVTALNDELNRIAETTSFGGNKLLAGTYGTKAMQIGADNGEAVMLSLKDMRSDNVMMGGVSYQAEEGKDKNWNVAAGDNDLTIALTDSFGNEQEIEINAKAGDDIEELATYINGQTDLVKASVGEGGKLQIFAGNNKVQGEIAFSGSLAGELGLGEGKNVTVDTIDVTTVQGAQESVAIVDAALKYVDSHRAELGAFQNRFNHAISNLDNINENVNASKSRIKDTDFAKETTQLTKTQILSQASSSILAQAKQAPNSALSLLG

SEQ ID NO: 17 - protein, 377 aa, synthetic construct
MAVNVNTNVAAMTAQRYLNNANSAQQTSMERLSSGFKINSAKDDAAGLQISNRLNVQSRGLDVAVRNANDGISIAQTAEGAMNETTNILQRMRDLSLQSANGSNSKSERVAIQEEVTALNDELNRIAETTSFGGNKLLNGTYGTKAMQIGADNGEAVMLSLKDMRSDNVMMGGVSYQAEEGKDKNWNVAAGDNDLTIALTDSFGNEQEIEINAKAGDDIEELATYINGQTDLVKASVGEGGKLQIFAGNNKVQGEIAFSGSLAGELGLGEGKAVTVDTIDVTTVQGAQESVAIVDAALKYVDSHRAELGAFQNRFNHAISNLDNINENVNASKSRIKDTDFAKETTQLTKTQILSQASSSILAQAKQAPNSALSLLG

SEQ ID NO: 18 - protein, 377 aa, synthetic construct
MAVNVNTNVAAMTAQRYLNNANSAQQTSMERLSSGFKINSAKDDAAGLQISNRLNVQSRGLDVAVRNANDGISIAQTAEGAMNETTNILQRMRDLSLQSANGSNSKSERVAIQEEVTALNDELNRIAETTSFGGNKLLNGTYGTKAMQIGADNGEAVMLSLKDMRSDNVMMGGVSYQAEEGKDKNWNVAAGDNDLTIALTDSFGNEQEIEINAKAGDDIEELATYINGQTDLVKASVGEGGKLQIFAGNNKVQGEIAFSGSLAGELGLGEGKNVTVDTIDVTTVQGAQESVAIVDAALKYVDSHRAELGAFQNRFNHAISNLDNINENVAASKSRIKDTDFAKETTQLTKTQILSQASSSILAQAKQAPNSALSLLG

SEQ ID NO: 19 - protein, 377 aa, synthetic construct
MAVNVNTNVAAMTAQRYLNNANSAQQTSMERLSSGFKINSAKDDAAGLQISNRLNVQSRGLDVAVRNANDGISIAQTAEGAMAETTNILQRMRDLSLQSAAGSNSKSERVAIQEEVTALNDELNRIAETTSFGGNKLLNGTYGTKAMQIGADNGEAVMLSLKDMRSDNVMMGGVSYQAEEGKDKNWNVAAGDNDLTIALTDSFGNEQEIEINAKAGDDIEELATYINGQTDLVKASVGEGGKLQIFAGNNKVQGEIAFSGSLAGELGLGEGKNVTVDTIDVTTVQGAQESVAIVDAALKYVDSHRAELGAFQNRFNHAISNLDNINENVNASKSRIKDTDFAKETTQLTKTQILSQASSSILAQAKQAPNSALSLLG

SEQ ID NO: 20 - protein, 377 aa, synthetic construct
MAVNVNTNVAAMTAQRYLNNANSAQQTSMERLSSGFKINSAKDDAAGLQISNRLNVQSRGLDVAVRNANDGISIAQTAEGAMAETTNILQRMRDLSLQSAAGSNSKSERVAIQEEVTALNDELNRIAETTSFGGNKLLAGTYGTKAMQIGADNGEAVMLSLKDMRSDNVMMGGVSYQAEEGKDKNWNVAAGDNDLTIALTDSFGNEQEIEINAKAGDDIEELATYINGQTDLVKASVGEGGKLQIFAGNNKVQGEIAFSGSLAGELGLGEGKNVTVDTIDVTTVQGAQESVAIVDAALKYVDSHRAELGAFQNRFNHAISNLDNINENVNASKSRIKDTDFAKETTQLTKTQILSQASSSILAQAKQAPNSALSLLG

SEQ ID NO: 21 - protein, 377 aa, synthetic construct
MAVNVNTNVAAMTAQRYLNNANSAQQTSMERLSSGFKINSAKDDAAGLQISNRLNVQSRGLDVAVRNANDGISIAQTAEGAMAETTNILQRMRDLSLQSAAGSNSKSERVAIQEEVTALNDELNRIAETTSFGGNKLLAGTYGTKAMQIGADNGEAVMLSLKDMRSDNVMMGGVSYQAEEGKDKNWNVAAGDNDLTIALTDSFGNEQEIEINAKAGDDIEELATYINGQTDLVKASVGEGGKLQIFAGNNKVQGEIAFSGSLAGELGLGEGKAVTVDTIDVTTVQGAQESVAIVDAALKYVDSHRAELGAFQNRFNHAISNLDNINENVNASKSRIKDTDFAKETTQLTKTQILSQASSSILAQAKQAPNSALSLLG

SEQ ID NO: 22 - protein, 377 aa, synthetic construct
MAVNVNTNVAAMTAQRYLNNANSAQQTSMERLSSGFKINSAKDDAAGLQISNRLNVQSRGLDVAVRNANDGISIAQTAEGAMAETTNILQRMRDLSLQSAAGSNSKSERVAIQEEVTALNDELNRIAETTSFGGNKLLAGTYGTKAMQIGADNGEAVMLSLKDMRSDNVMMGGVSYQAEEGKDKNWNVAAGDNDLTIALTDSFGNEQEIEINAKAGDDIEELATYINGQTDLVKASVGEGGKLQIFAGNNKVQGEIAFSGSLAGELGLGEGKAVTVDTIDVTTVQGAQESVAIVDAALKYVDSHRAELGAFQNRFNHAISNLDNINENVAASKSRIKDTDFAKETTQLTKTQILSQASSSILAQAKQAPNSALSLLG

SEQ ID NO: 23 - protein, 377 aa, synthetic construct
MAVNVNTNVAAMTAQRYLNNANSAQQTSMERLSSGFKINSAKDDAAGLQISNRLNVQSRGLDVAVRNANDGISIAQTAEGAMNETTNILQRMRDLSLQSANGSNSKSERVAIQEEVTALNDELNRIAETTSFGGNKLLAGTYGTKAMQIGADNGEAVMLSLKDMRSDNVMMGGVSYQAEEGKDKNWNVAAGDNDLTIALTDSFGNEQEIEINAKAGDDIEELATYINGQTDLVKASVGEGGKLQIFAGNNKVQGEIAFSGSLAGELGLGEGKAVTVDTIDVTTVQGAQESVAIVDAALKYVDSHRAELGAFQNRFNHAISNLDNINENVAASKSRIKDTDFAKETTQLTKTQILSQASSSILAQAKQAPNSALSLLG